European Patent Application EP 4 410 804 A1, published August 7, 2024. Title: Nucleic acid strand break method, nucleic acid strand break device, double-stranded DNA production method and double-stranded DNA production device. Applicant: 国立研究開発法人科学技術振興機構. Application WO. The sequence listing filed with the application follows.

SEQUENCE LISTING (24 sequences)

SEQ ID NO: 1 - DNA, 20 bp, artificial sequence
  source 1..20: mol_type = other DNA
  misc_feature 5: note = 3' thiolated nucleotide
  misc_feature 20: note = FAM bound at the 3' end
taactcacattaattgcgtt

SEQ ID NO: 2 - DNA, 20 bp, artificial sequence
  source 1..20: mol_type = other DNA
aacgcaattaatgtgagtta

SEQ ID NO: 3 - DNA, 41 bp, artificial sequence
  source 1..41: mol_type = other DNA
  misc_feature 15: note = 3' thiolated nucleotide
aggggtgcctaatgtgtgagctaactcacattaattgcgtt

SEQ ID NO: 4 - DNA, 22 bp, artificial sequence
  source 1..22: mol_type = other DNA
  misc_feature 1: note = FAM bound at the 5' end
aacgcaattaatgtgagttagc

SEQ ID NO: 5 - DNA, 41 bp, artificial sequence; identical to SEQ ID NO: 3
  source 1..41: mol_type = other DNA

SEQ ID NO: 6 - DNA, 27 bp, artificial sequence
  source 1..27: mol_type = other DNA
tgtgagctaactcacattaattgcgtt

SEQ ID NO: 7 - DNA, 15 bp, artificial sequence
  source 1..15: mol_type = other DNA
  misc_feature 15: note = FAM bound at the 3' end
cacattaattgcgtt

SEQ ID NO: 8 - DNA, 15 bp, artificial sequence
  source 1..15: mol_type = other DNA
  misc_feature 15: note = 3' thiolated nucleotide
aggggtgcctaatgt

SEQ ID NO: 9 - DNA, 26 bp, artificial sequence
  source 1..26: mol_type = other DNA
gtgagctaactcacattaattgcgtt

SEQ ID NO: 10 - DNA, 76 bp, artificial sequence
  source 1..76: mol_type = other DNA
cgcggatcctaatacgactcactatagggatccgaaggagatataccaatgtcgtttactttgaccaacaagaacg

SEQ ID NO: 11 - DNA, 20 bp, artificial sequence
  source 1..20: mol_type = other DNA
  misc_feature 8: note = 3' thiolated nucleotide
agcgccattcgccattcagg

SEQ ID NO: 12 - DNA, 20 bp, artificial sequence
  source 1..20: mol_type = other DNA
atggcgctttgcctggtttc

SEQ ID NO: 13 - DNA, 32 bp, artificial sequence
  source 1..32: mol_type = other DNA
ggctacggtctcacagcgcggctgaaatcatc

SEQ ID NO: 14 - DNA, 800 bp, artificial sequence
  source 1..800: mol_type = other DNA
atgtcgtttactttgaccaacaagaacgtgattttcgttgccggtctgggaggcattggtctggacaccagcaaggagctgctcaagcgcgatcccgtcgttttacaacgtcgtgactgggaaaaccctggcgttacccaacttaatcgccttgcagcacatccccctttcgccagctggcgtaatagcgaagaggcccgcaccgatcgcccttcccaacagttgcgcagcctgaatggcgaatggcgctttgcctggtttccggcaccagaagcggtgccggaaagctggctggagtgcgatcttcctgaggccgatactgtcgtcgtcccctcaaactggcagatgcacggttacgatgcgcccatctacaccaacgtaacctatcccattacggtcaatccgccgtttgttcccacggagaatccgacgggttgttactcgctcacatttaatgttgatgaaagctggctacaggaaggccagacgcgaattatttttgatggcgttaactcggcgtttcatctgtggtgcaacgggcgctgggtcggttacggccaggacagtcgtttgccgtctgaatttgacctgagcgcatttttacgcgccggagaaaaccgcctcgcggtgatggtgctgcgttggagtgacggcagttatctggaagatcaggatatgtggcggatgagcggcattttccgtgacgtctcgttgctgcataaaccgactacacaaatcagcgatttccatgttgccactcgctttaatgatgatttcagccgcgctgtgagaccgtagcc

SEQ ID NO: 15 - DNA, 52 bp, artificial sequence
  source 1..52: mol_type = other DNA
  misc_feature 15: note = 3' thiolated nucleotide
  misc_feature 31: note = 3' thiolated nucleotide
  misc_feature 51: note = 3' thiolated nucleotide
atgaaacgccgagttaacgccatcaaaaaataattcgcgtctggccttcctg

SEQ ID NO: 16 - DNA, 55 bp, artificial sequence
  source 1..55: mol_type = other DNA
  misc_feature 10: note = 3' thiolated nucleotide
  misc_feature 26: note = 3' thiolated nucleotide
  misc_feature 34: note = 3' thiolated nucleotide
  misc_feature 18: note = 3' thiolated nucleotide
agaattcaatgcccaaatgcccaaataaagctttaattcgcgtctggccttcctg

SEQ ID NO: 17 - DNA, 54 bp, artificial sequence
  source 1..54: mol_type = other DNA
  misc_feature 10: note = 3' thiolated nucleotide
  misc_feature 18: note = 3' thiolated nucleotide
  misc_feature 26: note = 3' thiolated nucleotide
  misc_feature 34: note = 3' thiolated nucleotide
aaagctttatttgggcatttgggcattgaattctggcgtttcatctgtggtgca

SEQ ID NO: 18 - DNA, 55 bp, artificial sequence; identical to SEQ ID NO: 16
  source 1..55: mol_type = other DNA
  misc_feature 18: note = 3' thiolated nucleotide
  misc_feature 34: note = 3' thiolated nucleotide

SEQ ID NO: 19 - DNA, 54 bp, artificial sequence; identical to SEQ ID NO: 17
  source 1..54: mol_type = other DNA
  misc_feature 18: note = 3' thiolated nucleotide
  misc_feature 34: note = 3' thiolated nucleotide

SEQ ID NO: 20 - DNA, 37 bp, artificial sequence
  source 1..37: mol_type = other DNA
attaaagctttatttgggcatttgggcattgaattct

SEQ ID NO: 21 - DNA, 37 bp, artificial sequence
  source 1..37: mol_type = other DNA
  misc_feature 10: note = 3' thiolated nucleotide
  misc_feature 18: note = 3' thiolated nucleotide
  misc_feature 26: note = 3' thiolated nucleotide
  misc_feature 34: note = 3' thiolated nucleotide
agaattcaatgcccaaatgcccaaataaagctttaat

SEQ ID NO: 22 - DNA, 37 bp, artificial sequence
  source 1..37: mol_type = other DNA
  misc_feature 10: note = 3' thiolated nucleotide
  misc_feature 18: note = 3' thiolated nucleotide
  misc_feature 26: note = 3' thiolated nucleotide
  misc_feature 34: note = 3' thiolated nucleotide
aaagctttatttgggcatttgggcattgaattctggc

SEQ ID NO: 23 - DNA, 37 bp, artificial sequence
  source 1..37: mol_type = other DNA
gccagaattcaatgcccaaatgcccttataaagcttt

SEQ ID NO: 24 - DNA, 802 bp, artificial sequence
  source 1..802: mol_type = other DNA
atgtcgtttactttgaccaacaagaacgtgattttcgttgccggtctgggaggcattggtctggacaccagcaaggagctgctcaagcgcgatcccgtcgttttacaacgtcgtgactgggaaaaccctggcgttacccaacttaatcgccttgcagcacatccccctttcgccagctggcgtaatagcgaagaggcccgcaccgatcgcccttcccaacagttgcgcagcctgaatggcgaatggcgctttgcctggtttccggcaccagaagcggtgccggaaagctggctggagtgcgatcttcctgaggccgatactgtcgtcgtcccctcaaactggcagatgcacggttacgatgcgcccatctacaccaacgtaacctatcccattacggtcaatccgccgtttgttcccacggagaatccgacgggttgttactcgctcacatttaatgttgatgaaagctggctacaggaaggccagacgcgaattaaagctttatttgggcatttgggcattgaattctggcgtttcatctgtggtgcaacgggcgctgggtcggttacggccaggacagtcgtttgccgtctgaatttgacctgagcgcatttttacgcgccggagaaaaccgcctcgcggtgatggtgctgcgttggagtgacggcagttatctggaagatcaggatatgtggcggatgagcggcattttccgtgacgtctcgttgctgcataaaccgactacacaaatcagcgatttccatgttgccactcgctttaatgatgatttcagccgcgctgt